European Patent Application EP 4 782 062 A2, published July 29, 2026. Title: NOVEL TRICYCLIC COMPOUNDS. Applicant: AbbVie Inc. Application WO PCT/US2010/058572, filed December 1, 2010. The sequence listing filed with the application follows.

SEQUENCE LISTING (5 sequences)

SEQ ID NO: 1 - protein, 18 aa, synthetic construct
  REGION 1..18: note = oligopeptide
  SITE 1: note = misc_feature - Bioin-(Ahx)-Alanin
  SITE 18: note = misc_feature - Arginine-amide
XGAGDQTPTPTRFLKRPX

SEQ ID NO: 2 - protein, 12 aa, synthetic construct
  REGION 1..12: note = oligopeptide
  SITE 1: note = misc_feature - Biotin-(Ahx)-Glycine
XAEEEIYAAFFA

SEQ ID NO: 3 - protein, 10 aa, synthetic construct
  REGION 1..10: note = oligopeptide
  SITE 1: note = misc_feature - Biotin-(Ahx)-Alanine
  SITE 10: note = misc_feature - Alanine-amide
XEEEYFFLFX

SEQ ID NO: 4 - protein, 25 aa, synthetic construct
  REGION 1..25: note = oligopeptide
  SITE 1: note = misc_feature - Biotin-(Ahx)-Valine
  SITE 25: note = misc_feature - Arginine-amide
XHFFKNIVTPRTPPPSQGKGAEGQX

SEQ ID NO: 5 - protein, 8 aa, synthetic construct
  REGION 1..8: note = oligopeptide
DYKDDDDK